European Patent Application EP 4 692 310 A1, published February 11, 2026. Title: 신규한 바실러스 메가테리움 HyangYak-01 균주 및 이의 용도. Applicant: 코스맥스 주식회사. The sequence listing filed with the application follows.

SEQUENCE LISTING (3 sequences)

SEQ ID NO: 1 - DNA, 1429 bp, Bacillus megaterium
  source 1..1429: mol_type = genomic DNA
ctatctgcagtcgagcgactgattagaagcttgcttctatgacgttagcggcggacgggtgagtaacacgtgggcaacctgcctgtaagactgggataacttcgggaaaccgaagctaataccggataggatcttctccttcatgggagatgattgaaagatggtttcggctatcacttacagatgggcccgcggtgcattagctagttggtgaggtaacggctcaccaaggccacgatgcatagccgacctgagagggtgatcggccacactgggactgagacacggcccagactcctacgggaggcagcagtagggaatcttccgcaatggacgaaagtctgacggagcaacgccgcgtgagtgatgaaggctttcgggtcgtaaaactctgttgttagggaagaacaagtacaagagtaactgcttgtaccttgacggtacctaaccagaaagccacggctaactacgtgccagcagccgcggtaatacgtaggtggcaagcgttatccggaattattgggcgtaaagcgcgcgcaggcggtttcttaagtctgatgtgaaagcccacggctcaaccgtggagggtcattggaaactggggaacttgagtgcagaagagaaaagcggaattccacgtgtagcggtgaaatgcgtagagatgtggaggaacaccagtggcgaaggcggctttttggtctgtaactgacgctgaggcgcgaaagcgtggggagcaaacaggattagataccctggtagtccacgccgtaaacgatgagtgctaagtgttagagggtttccgccctttagtgctgcagctaacgcattaagcactccgcctggggagtacggtcgcaagactgaaactcaaaggaattgacgggggcccgcacaagcggtggagcatgtggtttaattcgaagcaacgcgaagaaccttaccaggtcttgacatcctctgacaactctagagatagagcgttccccttcgggggacagagtgacaggtggtgcatggttgtcgtcagctcgtgtcgtgagatgttgggttaagtcccgcaacgagcgcaacccttgatcttagttgccagcatttagttgggcactctaaggtgactgccggtgacaaaccggaggaaggtggggatgacgtcaaatcatcatgccccttatgacctgggctacacacgtgctacaatggatggtacaaagggctgcaagaccgcgaggtcaagccaatcccataaaaccattctcagttcggattgtaggctgcaactcgcctacatgaagctggaatcgctagtaatcgcggatcagcatgccgcggtgaatacgttcccgggccttgtacacaccgcccgtcacaccacgagagtttgtaacacccgaagtcggtggagtaaccgtaaggagctagccgccaagtg

SEQ ID NO: 2 - DNA, 20 bp, synthetic construct
  source 1..20: mol_type = other DNA
agagtttgatcmtggctcag

SEQ ID NO: 3 - DNA, 20 bp, synthetic construct
  source 1..20: mol_type = other DNA
ggttaccttgttacgacttc